European Patent Specification EP 3 556 771 B1, published October 2, 2024. Title: Antibody. Applicant: OSAKA UNIVERSITY. The sequence listing filed with the application follows.

SEQUENCE LISTING (99 sequences)

SEQ ID NO: 1 - protein, 7 aa, Artificial Sequence
  2B12 heavy chain CDR1
GYTFTRF

SEQ ID NO: 2 - protein, 6 aa, Artificial Sequence
  2B12 heavy chain CDR2
YPGSGD

SEQ ID NO: 3 - protein, 13 aa, Artificial Sequence
  2B12 heavy chain CDR3
WGIYYGNPYAMDY

SEQ ID NO: 4 - protein, 122 aa, Artificial Sequence
  2B12 Heavy chain variable region
QVQLQQSGAELARPGASVKLSCKASGYTFTRFGMSWVKQRTGQGLEWIGEIYPGSGDTYYSENFKGKATLTADKSSGTAYMELRSLTSEDSAVYFCARWGIYYGNPYAMDYWGQGTSVTVSS

SEQ ID NO: 5 - protein, 16 aa, Artificial Sequence
  2B12 light chain CDR1
RSSKSLLHSNGNTYLY

SEQ ID NO: 6 - protein, 7 aa, Artificial Sequence
  2B12 light chain CDR2
RMSNLAS

SEQ ID NO: 7 - protein, 9 aa, Artificial Sequence
  2B12 light chain CDR3
LQHLEYPFT

SEQ ID NO: 8 - protein, 114 aa, Artificial Sequence
  2B12 light chain variable region
DIVMTQAAPSVPVTPGESVSISCRSSKSLLHSNGNTYLYWFLQRPGQSPQLLIYRMSNLASGVPDRFSGSGSGTAFTLRISRVEAEDVGVYYCLQHLEYPFTFGSGTKLEIKRA

SEQ ID NO: 9 - protein, 7 aa, Artificial Sequence
  2B1 heavy chain CDR1
GYTFTTF

SEQ ID NO: 10 - protein, 6 aa, Artificial Sequence
  2B1 heavy chain CDR2
APYSGG

SEQ ID NO: 11 - protein, 11 aa, Artificial Sequence
  2B1 heavy chain CDR3
WDFTYGSNLDY

SEQ ID NO: 12 - protein, 120 aa, Artificial Sequence
  2B1 Heavy chain variable region
QVQLQQPGAELVKPGASVKLSCKASGYTFTTFWIHWVKQRPGRGLEWIGRIAPYSGGTTYNEKFKSKATLTVDRPSTTAYMQLISLTSEDSAVYYCARWDFTYGSNLDYWGQGTTLTVSS

SEQ ID NO: 13 - protein, 11 aa, Artificial Sequence
  2B1 light chain CDR1
KASQNVRTAVA

SEQ ID NO: 14 - protein, 7 aa, Artificial Sequence
  2B1 light chain CDR2
LASNRHT

SEQ ID NO: 15 - protein, 9 aa, Artificial Sequence
  2B1 light chain CDR3
LGHWDYPYT

SEQ ID NO: 16 - protein, 109 aa, Artificial Sequence
  2B1 light chain variable region
DIVMTQSQKFMSTSVGDRVSIPCKASQNVRTAVAWYQQKPGQSPKALIYLASNRHTGVPDRFTGSGSGTDFTLTISNVQSEDLADYFCLGHWDYPYTFGGGTKLEIKRA

SEQ ID NO: 17 - protein, 7 aa, Artificial Sequence
  4F1 heavy chain CDR1
GYSFTSY

SEQ ID NO: 18 - protein, 6 aa, Artificial Sequence
  4F1 heavy chain CDR2
YPGSGN

SEQ ID NO: 19 - protein, 12 aa, Artificial Sequence
  4F1 heavy chain CDR3
PYYGSRRDYFDY

SEQ ID NO: 20 - protein, 121 aa, Artificial Sequence
  4F1 Heavy chain variable region
QVQLQQSGPELVKPGASVKISCKASGYSFTSYYIHWVKQRPGQGLEWIGWIYPGSGNTKYNEKFKGKATLTADTSSSTAYMQLSSLTSEDSAVYYCASPYYGSRRDYFDYWGQGTTLTVSS

SEQ ID NO: 21 - protein, 17 aa, Artificial Sequence
  4F1 light chain CDR1
KSSQSLLYSSNQKNYLA

SEQ ID NO: 22 - protein, 7 aa, Artificial Sequence
  4F1 light chain CDR2
WASTRES

SEQ ID NO: 23 - protein, 9 aa, Artificial Sequence
  4F1 light chain CDR3
QQYYSYPLT

SEQ ID NO: 24 - protein, 115 aa, Artificial Sequence
  4F1 light chain variable region
DIVMSQSPSSLAVSVGEKVTMSCKSSQSLLYSSNQKNYLAWYQQKPGQSPKLLIYWASTRESGVPDRFTGSGSGTDFTLTISSVKAEDLAVYYCQQYYSYPLTFGAGTKLELKRA

SEQ ID NO: 25 - protein, 8 aa, Artificial Sequence
  4D2 heavy chain CDR1
GYSITSGY

SEQ ID NO: 26 - protein, 5 aa, Artificial Sequence
  4D2 heavy chain CDR2
SYDGS

SEQ ID NO: 27 - protein, 10 aa, Artificial Sequence
  4D2  heavy chain CDR3
EAYYSNYGFS

SEQ ID NO: 28 - protein, 119 aa, Artificial Sequence
  4D2 Heavy chain variable region
DVQLQESGPGLVKPSQSLSLTCSVTGYSITSGYYWNWIRQFPGNKLEWMGYISYDGSNNYNPSLKNRISITRDTSKNQFFLKLNSVTTEDTATYYCAREAYYSNYGFSPGQGTLVTVSA

SEQ ID NO: 29 - protein, 17 aa, Artificial Sequence
  4D2 light chain CDR1
KSSQSLLYSSNQKNYLA

SEQ ID NO: 30 - protein, 7 aa, Artificial Sequence
  4D2 light chain CDR2
WASTRES

SEQ ID NO: 31 - protein, 9 aa, Artificial Sequence
  4D2 light chain CDR3
QQYYRYPYT

SEQ ID NO: 32 - protein, 115 aa, Artificial Sequence
  4D2 light chain variable region
DIVMSQSPSSLAVSVGEKVTMSCKSSQSLLYSSNQKNYLAWYQQKPGQSPKLLIYWASTRESGVPDRFTGSGSGTDFTLTISSVKAEDLAVYYCQQYYRYPYTFGGGTKLEIKRA

SEQ ID NO: 33 - protein, 7 aa, Artificial Sequence
  1B3 heavy chain CDR1
GYSFTAH

SEQ ID NO: 34 - protein, 6 aa, Artificial Sequence
  1B3 heavy chain CDR2
NTYSGV

SEQ ID NO: 35 - protein, 9 aa, Artificial Sequence
  1B3 heavy chain CDR3
SHYDRKFGY

SEQ ID NO: 36 - protein, 118 aa, Artificial Sequence
  1B3 Heavy chain variable region
QIQLVQSGPELKKPGETVKISCKASGYSFTAHGMSWVKQAPGKGLKWMGWINTYSGVPAYADDFKGRFAFSLETSPSTAFLQINNLKNEDTATYFCTRSHYDRKFGYWGQGTLVTVSA

SEQ ID NO: 37 - protein, 14 aa, Artificial Sequence
  1B3 light chain CDR1
RSSTGAVTTSNYAN

SEQ ID NO: 38 - protein, 7 aa, Artificial Sequence
  1B3 light chain CDR2
DTNNRAP

SEQ ID NO: 39 - protein, 9 aa, Artificial Sequence
  1B3 light chain CDR3
ALWYSNLWV

SEQ ID NO: 40 - protein, 112 aa, Artificial Sequence
  1B3 light chain variable region
QAVVTQESALTTSPGETVTLTCRSSTGAVTTSNYANWVQEKPDHLFTGLIGDTNNRAPGVPARFSGSLIGDKAALTITGAQTGDEAIYFCALWYSNLWVFGGGTKLTVRGQP

SEQ ID NO: 41 - protein, 7 aa, Artificial Sequence
  1D1 heavy chain CDR1
GYTFTTY

SEQ ID NO: 42 - protein, 6 aa, Artificial Sequence
  1D1 heavy chain CDR2
APNSGG

SEQ ID NO: 43 - protein, 11 aa, Artificial Sequence
  1D1 heavy chain CDR3
WDFTFGTNLDY

SEQ ID NO: 44 - protein, 120 aa, Artificial Sequence
  1D1 Heavy chain variable region
QVQLQQPGAEHVKPGASVKLSCKASGYTFTTYWIHWVKQRPGRGLEWIGRIAPNSGGTKYNENFKSKATLTVDRPSTTAYMQLSGLTSEDSAVYYCARWDFTFGTNLDYWGQGTTLTVSS

SEQ ID NO: 45 - protein, 11 aa, Artificial Sequence
  1D1 light chain CDR1
KASQNVRTAVA

SEQ ID NO: 46 - protein, 7 aa, Artificial Sequence
  1D1 light chain CDR2
LASNRHT

SEQ ID NO: 47 - protein, 9 aa, Artificial Sequence
  1D1 light chain CDR3
LQHWTYPYT

SEQ ID NO: 48 - protein, 109 aa, Artificial Sequence
  1D1 light chain variable region
DIVMTQSQKFMSTSVGDRVSITCKASQNVRTAVAWYQQKPGQSPKALIFLASNRHTGVPDRFTGSGSGTDFTLTITNVQSEDLADYFCLQHWTYPYTFGGGTKLEIKRA

SEQ ID NO: 49 - protein, 7 aa, Artificial Sequence
  3A5 heavy chain CDR1
GYTFTSY

SEQ ID NO: 50 - protein, 6 aa, Artificial Sequence
  3A5 heavy chain CDR2
NPSNGG

SEQ ID NO: 51 - protein, 13 aa, Artificial Sequence
  3A5 heavy chain CDR3
YYGSSFLYWYFDV

SEQ ID NO: 52 - protein, 122 aa, Artificial Sequence
  3A5 Heavy chain variable region
QVQLQQPGTELVKPGASVKLSCKASGYTFTSYWMHWVKQRPGQGLEWIGNINPSNGGTNYNEKFKSKATLTVDKSSTTAYMLLSSLTSEDSAVYYCARYYGSSFLYWYFDVWGTGTTVTVSS

SEQ ID NO: 53 - protein, 11 aa, Artificial Sequence
  3A5 light chain CDR1
KASQDVGTAVA

SEQ ID NO: 54 - protein, 7 aa, Artificial Sequence
  3A5 light chain CDR2
WASTRHT

SEQ ID NO: 55 - protein, 8 aa, Artificial Sequence
  3A5 light chain CDR3
QQYSSYPT

SEQ ID NO: 56 - protein, 108 aa, Artificial Sequence
  3A5 light chain variable region
DIVMTQSHKFMSSSVGDRVSITCKASQDVGTAVAWYQQKPGQSPKILIYWASTRHTGVPDRFTGSGSGTDFTLTISNVQSEDLADYFCQQYSSYPTFGSGTKLEIKRA

SEQ ID NO: 57 - protein, 7 aa, Artificial Sequence
  2D1 heavy chain CDR1
GYTFTSY

SEQ ID NO: 58 - protein, 6 aa, Artificial Sequence
  2D1 heavy chain CDR2
DPNSGG

SEQ ID NO: 59 - protein, 6 aa, Artificial Sequence
  2D1 heavy chain CDR3
WGTGDY

SEQ ID NO: 60 - protein, 115 aa, Artificial Sequence
  2D1 Heavy chain variable region
QVQLQQPGAELVKPGASVKLSCKASGYTFTSYWMHWVKQRPGRGLEWIGRIDPNSGGTKYNEKFKSKATLTVDKPSSTAYMQLSSLTSEDSAVYYCARWGTGDYWGQGTTLTVSS

SEQ ID NO: 61 - protein, 15 aa, Artificial Sequence
  2D1 light chain CDR1
RASKSVSTSGYSYMH

SEQ ID NO: 62 - protein, 7 aa, Artificial Sequence
  2D1 light chain CDR2
LASNLES

SEQ ID NO: 63 - protein, 9 aa, Artificial Sequence
  2D1 light chain CDR3
QHSRELPFT

SEQ ID NO: 64 - protein, 113 aa, Artificial Sequence
  2D1 light chain variable region
DIVLTQSPASLAVSLGQRATISCRASKSVSTSGYSYMHWYQQKPGQPPKLLIYLASNLESGVPARFSGSGSGTDFTLNIHPVEEEDAATYYCQHSRELPFTFGSGTKLEIKRA

SEQ ID NO: 65 - protein, 7 aa, Artificial Sequence
  4A1 heavy chain CDR1
GYTFTSY

SEQ ID NO: 66 - protein, 6 aa, Artificial Sequence
  4A1 heavy chain CDR2
YPRSGN

SEQ ID NO: 67 - protein, 8 aa, Artificial Sequence
  4A1 heavy chain CDR3
PYEGYFDY

SEQ ID NO: 68 - protein, 117 aa, Artificial Sequence
  4A1 Heavy chain variable region
QVQLQQSGAELARPGASVKLSCKASGYTFTSYGISWVNQRTGQGLEWIGEIYPRSGNTYFNEKFQGKATLTADKSSSTAYMELRSLTSEDSAVFFCARPYEGYFDYWGQGTTLTVSS

SEQ ID NO: 69 - protein, 15 aa, Artificial Sequence
  4A1 light chain CDR1
RASKSVSTSGYSYMH

SEQ ID NO: 70 - protein, 7 aa, Artificial Sequence
  4A1 light chain CDR2
LASNLES

SEQ ID NO: 71 - protein, 9 aa, Artificial Sequence
  4A1 light chain CDR3
QHSRELPFT

SEQ ID NO: 72 - protein, 113 aa, Artificial Sequence; identical to SEQ ID NO: 64
  4A1 light chain variable region

SEQ ID NO: 73 - protein, 218 aa, Homo sapiens
MGSAALEILGLVLCLVGWGGLILACGLPMWQVTAFLDHNIVTAQTTWKGLWMSCVVQSTGHMQCKVYDSVLALSTEVQAARALTVSAVLLAFVALFVTLAGAQCTTCVAPGPAKARVALTGGVLYLFCGLLALVPLCWFANIVVREFYDPSVPVSQKYELGAALYIGWAATALLMVGGCLLCCGAWVCTGRPDLSFPVKYSAPRRPTATGDYDKKNYV

SEQ ID NO: 74 - DNA, 657 bp, Artificial Sequence
  human Claudin 5 coding sequence
atgggatctgctgctcttgagatccttggacttgttctctgccttgttggatggggaggacttatccttgcttgcggacttcctatgtggcaggttacagctttcctcgatcacaacatcgtgactgctcagactacttggaagggactctggatgtcttgcgtggtgcaatctactggacacatgcagtgcaaggtgtacgattctgttctcgctctctctactgaggttcaagctgctagggctcttactgtttctgctgttctcctcgctttcgtggctctcttcgttactcttgctggtgctcagtgtactacctgtgttgctcctggacctgctaaggctagagttgctcttacaggtggtgtgctctaccttttctgtggacttcttgctcttgtgcctctctgctggttcgctaacatcgtggttagagagttctacgatccttctgtgcctgtgtctcagaagtacgaacttggagctgctctctacattggatgggctgctactgctctccttatggttggaggatgccttctttgttgtggtgcttgggtgtgcactggaaggcctgatttgtctttcccagtgaagtactctgctcctagaaggcctactgctaccggtgattacgataagaagaactacgtttga

SEQ ID NO: 75 - protein, 189 aa, Artificial Sequence
  human mouse-chimera Claudin 5
MGSAALEILGLVLCLVGWVGLILACGLPMWQVTAFLDHNIVTAQTTWKGLWMSCVVQSTGHMQCKVYDSVLALSTEVQAARALTVSAVLLALVALFVTLTGAQCTTCVAPGPVKARVALTGGALYAVCGLLALVPLCWFANIVVREFYDPSVPVSQKYELGAALYIGWAATALLMVGGGLVCCGAWVCT

SEQ ID NO: 76 - DNA, 570 bp, Artificial Sequence
  human mouse-chimera Claudin 5 coding sequence
atgggatctgctgctcttgagatccttggacttgttctctgcctcgttggatgggttggacttatccttgcttgcggacttcctatgtggcaggttacagctttcctcgatcacaacatcgtgactgctcagactacttggaagggactctggatgtcttgcgtggtgcaatctactggacacatgcagtgcaaggtgtacgattctgttctcgctctctctactgaggttcaagctgctagggctcttactgtttctgctgttctccttgctctcgtggctctcttcgttactcttactggtgctcagtgtactacctgtgttgctcctggacctgttaaggctagagttgctcttacaggtggtgctctctacgctgtttgtggacttcttgctcttgtgccactttgctggttcgctaacatcgtggtgagagagttctacgatccttctgtgcctgtgtctcagaagtacgaacttggagctgcactctacattggatgggctgctactgctctccttatggttggaggtggtcttgtttgttgtggtgcttgggtgtgcacttga

SEQ ID NO: 77 - protein, 282 aa, Artificial Sequence
  extracellular domain reversible Claudin 5
MGSAALEILGLVLCLVGWGGLILACGLPMWQVTAFLDHNIVTAQTTWKGLWMSCVVQSTGHMQCKVYDSVLALSTEVQAARALTVSAVLLAFWGGLILACGLPMWQVTAFLDHNIVTAQTTWKGLWMSCVVQSTGHMQCKVYDSVLALSTEVQAARALTVSAVLLAFLLALVPLCWFANIVVREFYDPSVPVSQKYELGAALYIGWAATALLMVGLLALVPLCWFANIVVREFYDPSVPVSQKYELGAALYIGWAATALLMVGWGGLILACGLPMWQVTAFL

SEQ ID NO: 78 - DNA, 849 bp, Artificial Sequence
  extracellular domain reversible Claudin 5 coding sequence
atgggatctgctgctcttgagatccttggacttgttctctgccttgttggatggggaggacttatccttgcttgcggacttcctatgtggcaggttacagctttcctcgatcacaacatcgtgactgctcagactacttggaagggactctggatgtcttgcgtggtgcaatctactggacacatgcagtgcaaggtgtacgattctgttctcgctctctctactgaggttcaagctgctagggctcttactgtttctgctgttcttctcgctttctggggtggtctgatcctggcctgtggcctgccaatgtggcaagtgaccgccttcctggaccataatatagtcaccgcccagaccacctggaaaggcctgtggatgagctgtgtcgtccagagcacaggccatatgcaatgtaaggtttatgacagcgtgctggccctgagcacagaagtgcaggcagcaagagccctgaccgtgagtgcagtgctgctggcctttttgctcgctcttgttccactctgctggttcgctaacattgtggtgagagagttctacgacccatccgttccagtgtctcagaagtatgaacttggcgctgctctctacattggatgggctgctactgctcttttgatggtgggattattggcactcgttccactctgttggtttgccaatattgttgtgcgtgaattttatgacccatcggtgccagtgtcgcaaaaatacgagttgggtgctgccttgtatatcggttgggcagctacagctcttttgatggtaggttggggtggacttattctcgcatgtggactcccaatgtggcaggttaccgcatttctttga

SEQ ID NO: 79 - protein, 211 aa, Homo sapiens
MANAGLQLLGFILAFLGWIGAIVSTALPQWRIYSYAGDNIVTAQAMYEGLWMSCVSQSTGQIQCKVFDSLLNLSSTLQATRALMVVGILLGVIAIFVATVGMKCMKCLEDDEVQKMRMAVIGGAIFLLAGLAILVATAWYGNRIVQEFYDPMTPVNARYEFGQALFTGWAAASLCLLGGALLCCSCPRKTTSYPTPRPYPKPAPSSGKDYV

SEQ ID NO: 80 - protein, 230 aa, Homo sapiens
MASLGLQLVGYILGLLGLLGTLVAMLLPSWKTSSYVGASIVTAVGFSKGLWMECATHSTGITQCDIYSTLLGLPADIQAAQAMMVTSSAISSLACIISVVGMRCTVFCQESRAKDRVAVAGGVFFILGGLLGFIPVAWNLHGILRDFYSPLVPDSMKFEIGEALYLGIISSLFSLIAGIILCFSCSSQRNRSNYYDAYQAQPLATRSSPRPGQPPKVKSEFNSYSLTGYV

SEQ ID NO: 81 - protein, 220 aa, Homo sapiens
MSMGLEITGTALAVLGWLGTIVCCALPMWRVSAFIGSNIITSQNIWEGLWMNCVVQSTGQMQCKVYDSLLALPQDLQAARALIVVAILLAAFGLLVALVGAQCTNCVQDDTAKAKITIVAGVLFLLAALLTLVPVSWSANTIIRDFYNPVVPEAQKREMGAGLYVGWAAAALQLLGGALLCCSCPPREKKYTATKVVYSAPRSTGPGASLGTGYDRKDYV

SEQ ID NO: 82 - protein, 209 aa, Homo sapiens
MASMGLQVMGIALAVLGWLAVMLCCALPMWRVTAFIGSNIVTSQTIWEGLWMNCVVQSTGQMQCKVYDSLLALPQDLQAARALVIISIIVAALGVLLSVVGGKCTNCLEDESAKAKTMIVAGVVFLLAGLMVIVPVSWTAHNIIQDFYNPLVASGQKREMGASLYVGWAASGLLLLGGGLLCCNCPPRTDKPYSAKYSAARSAAASNYV

SEQ ID NO: 83 - protein, 220 aa, Homo sapiens
MASAGMQILGVVLTLLGWVNGLVSCALPMWKVTAFIGNSIVVAQVVWEGLWMSCVVQSTGQMQCKVYDSLLALPQDLQAARALCVIALLVALFGLLVYLAGAKCTTCVEEKDSKARLVLTSGIVFVISGVLTLIPVCWTAHAIIRDFYNPLVAEAQKRELGASLYLGWAASGLLLLGGGLLCCTCPSGGSQGPSHYMARYSTSAPAISRGPSEYPTKNYV

SEQ ID NO: 84 - protein, 211 aa, Homo sapiens
MANSGLQLLGFSMALLGWVGLVACTAIPQWQMSSYAGDNIITAQAMYKGLWMDCVTQSTGMMSCKMYDSVLALSAALQATRALMVVSLVLGFLAMFVATMGMKCTRCGGDDKVKKARIAMGGGIIFIVAGLAALVACSWYGHQIVTDFYNPLIPTNIKYEFGPAIFIGWAGSALVILGGALLSCSCPGNESKAGYRVPRSYPKSNSSKEYV

SEQ ID NO: 85 - protein, 217 aa, Homo sapiens
MASTGLELLGMTLAVLGWLGTLVSCALPLWKVTAFIGNSIVVAQVVWEGLWMSCVVQSTGQMQCKVYDSLLALPQDLQAARALCVIALLLALLGLLVAITGAQCTTCVEDEGAKARIVLTAGVILLLAGILVLIPVCWTAHAIIQDFYNPLVAEALKRELGASLYLGWAAAALLMLGGGLLCCTCPPPQVERPRGPRLGYSIPSRSGASGLDKRDYV

SEQ ID NO: 86 - protein, 211 aa, Mus musculus
MANAGLQLLGFILASLGWIGSIVSTALPQWKIYSYAGDNIVTAQAIYEGLWMSCVSQSTGQIQCKVFDSLLNLNSTLQATRALMVIGILLGLIAIFVSTIGMKCMRCLEDDEVQKMWMAVIGGIIFLISGLATLVATAWYGNRIVQEFYDPLTPINARYEFGQALFTGWAAASLCLLGGVLLSCSCPRKTTSYPTPRPYPKPTPSSGKDYV

SEQ ID NO: 87 - protein, 230 aa, Mus musculus
MASLGVQLVGYILGLLGLLGTSIAMLLPNWRTSSYVGASIVTAVGFSKGLWMECATHSTGITQCDIYSTLLGLPADIQAAQAMMVTSSAMSSLACIISVVGMRCTVFCQDSRAKDRVAVVGGVFFILGGILGFIPVAWNLHGILRDFYSPLVPDSMKFEIGEALYLGIISALFSLVAGVILCFSCSPQGNRTNYYDGYQAQPLATRSSPRSAQQPKAKSEFNSYSLTGYV

SEQ ID NO: 88 - protein, 219 aa, Mus musculus
MSMGLEITGTSLAVLGWLCTIVCCALPMWRVSAFIGSSIITAQITWEGLWMNCVVQSTGQMQCKMYDSLLALPQDLQAARALIVVSILLAAFGLLVALVGAQCTNCVQDETAKAKITIVAGVLFLLAALLTLVPVSWSANTIIRDFYNPLVPEAQKREMGAGLYVGWAAAALQLLGGALLCCSCPPRDKYAPTKILYSAPRSTGPGTGTGTAYDRKDYV

SEQ ID NO: 89 - protein, 210 aa, Mus musculus
MASMGLQVLGISLAVLGWLGIILSCALPMWRVTAFIGSNIVTAQTSWEGLWMNCVVQSTGQMQCKMYDSMLALPQDLQAARALMVISIIVGALGMLLSVVGGKCTNCMEDETVKAKIMITAGAVFIVASMLIMVPVSWTAHNVIRDFYNPMVASGQKREMGASLYVGWAASGLLLLGGGLLCCSCPPRSNDKPYSAKYSAARSVPASNYV

SEQ ID NO: 90 - protein, 218 aa, Mus musculus
MGSAALEILGLVLCLVGWVGLILACGLPMWQVTAFLDHNIVTAQTTWKGLWMSCVVQSTGHMQCKVYESVLALSAEVQAARALTVGAVLLALVALFVTLTGAQCTTCVAPGPVKARVALTGGALYAVCGLLALVPLCWFANIVVREFYDPTVPVSQKYELGAALYIGWAASALLMCGGGLVCCGAWVCTGRPEFSFPVKYSAPRRPTANGDYDKKNYV

SEQ ID NO: 91 - protein, 218 aa, Rattus norvegicus
MGSAALEILGLVLCLVGWVGLILACGLPMWQVTAFLDHNIVTAQTTWKGLWMSCVVQSTGHMQCKVYESVLALSAEVQAARALTVGAVLLALVALFVTLTGAQCTTCVAPGPVKARVALTGGALYALCGLLALVPLCWFANIVVREFYDPTVPVSQKYELGAALYIGWAASALLMCGGGLVCCGAWVCTGRPEFSFPVKYSAPRRTTANGDYDKKNYV

SEQ ID NO: 92 - protein, 218 aa, Macaca fascicularis
MGSAALEILGLVLCLVGWGGLILACGLPMWQVTAFLDHNIVTAQTTWKGLWMSCVVQSTGHMQCKVYDSVLALSTEVQAARALTVGAVLLAFVALFVTLAGAQCTTCVAPGPAKARVALTGGVLYLLCGLLALVPLCWFANIVVREFYDPSVPVSQKYELGAALYIGWAATALLMVGGGLLCCGAWVCTSRPDLSFPVKYSAPRRPTATGDYDKKNYV

SEQ ID NO: 93 - protein, 218 aa, Artificial Sequence
  chimera claudin 1-1-5
MGSAALEILGLVLCLVGWGGLILACALPQWRIYSYAGDNIVTAQAMYEGLWMSCVSQSTGQIQCKVFDSLLNLSSTVQAARALTVSAVLLAFVALFVTLAGAQCTTCVAPGPAKARVALTGGVLYLFCGLLALVPLCWFANIVVREFYDPSVPVSQKYELGAALYIGWAATALLMVGGCLLCCGAWVCTGRPDLSFPVKYSAPRRPTATGDYDKKNYV

SEQ ID NO: 94 - protein, 218 aa, Artificial Sequence
  chimera claudin 1-5-5
MGSAALEILGLVLCLVGWGGLILACALPQWRIYSYAGDNIVTAQAMYEGLWMSCVVQSTGHMQCKVYDSVLALSTEVQAARALTVSAVLLAFVALFVTLAGAQCTTCVAPGPAKARVALTGGVLYLFCGLLALVPLCWFANIVVREFYDPSVPVSQKYELGAALYIGWAATALLMVGGCLLCCGAWVCTGRPDLSFPVKYSAPRRPTATGDYDKKNYV

SEQ ID NO: 95 - protein, 218 aa, Artificial Sequence
  chimera claudin 5-1-5
MGSAALEILGLVLCLVGWGGLILACGLPMWQVTAFLDHNIVTAQTTWKGLWMSCVSQSTGQIQCKVFDSLLNLSSTVQAARALTVSAVLLAFVALFVTLAGAQCTTCVAPGPAKARVALTGGVLYLFCGLLALVPLCWFANIVVREFYDPSVPVSQKYELGAALYIGWAATALLMVGGCLLCCGAWVCTGRPDLSFPVKYSAPRRPTATGDYDKKNYV

SEQ ID NO: 96 - protein, 218 aa, Artificial Sequence
  chimera claudin 5-5-1
MGSAALEILGLVLCLVGWGGLILACGLPMWQVTAFLDHNIVTAQTTWKGLWMSCVVQSTGHMQCKVYDSVLALSTEVQAARALTVSAVLLAFVALFVTLAGAQCTTCVAPGPAKARVALTGGVLYLFCGLLALVPLCWFANIVVREFYDPMTPVNARYEFGQALYIGWAATALLMVGGCLLCCGAWVCTGRPDLSFPVKYSAPRRPTATGDYDKKNYV

SEQ ID NO: 97 - protein, 218 aa, Artificial Sequence
  point mutated claudin 5 D68E
MGSAALEILGLVLCLVGWGGLILACGLPMWQVTAFLDHNIVTAQTTWKGLWMSCVVQSTGHMQCKVYESVLALSTEVQAARALTVSAVLLAFVALFVTLAGAQCTTCVAPGPAKARVALTGGVLYLFCGLLALVPLCWFANIVVREFYDPSVPVSQKYELGAALYIGWAATALLMVGGCLLCCGAWVCTGRPDLSFPVKYSAPRRPTATGDYDKKNYV

SEQ ID NO: 98 - protein, 218 aa, Artificial Sequence
  point mutated claudin 5 T75A
MGSAALEILGLVLCLVGWGGLILACGLPMWQVTAFLDHNIVTAQTTWKGLWMSCVVQSTGHMQCKVYDSVLALSAEVQAARALTVSAVLLAFVALFVTLAGAQCTTCVAPGPAKARVALTGGVLYLFCGLLALVPLCWFANIVVREFYDPSVPVSQKYELGAALYIGWAATALLMVGGCLLCCGAWVCTGRPDLSFPVKYSAPRRPTATGDYDKKNYV

SEQ ID NO: 99 - protein, 218 aa, Artificial Sequence
  point mutated claudin 5 S151T
MGSAALEILGLVLCLVGWGGLILACGLPMWQVTAFLDHNIVTAQTTWKGLWMSCVVQSTGHMQCKVYDSVLALSTEVQAARALTVSAVLLAFVALFVTLAGAQCTTCVAPGPAKARVALTGGVLYLFCGLLALVPLCWFANIVVREFYDPTVPVSQKYELGAALYIGWAATALLMVGGCLLCCGAWVCTGRPDLSFPVKYSAPRRPTATGDYDKKNYV